European Patent Application EP 4 653 459 A1, published November 26, 2025. Title: Antibody spcifically binding to IL-10 Receptor and use thereof. Applicant: IUCF-HYU. Application KR PCT/KR2023/021045, filed December 20, 2023. The sequence listing filed with the application follows.

SEQUENCE LISTING (4 sequences)

SEQ ID NO: 1 - protein, 578 aa, unidentified
MLPCLVVLLAALLSLRLGSDAHGTELPSPPSVWFEAEFFHHILHWTPIPNQSESTCYEVALLRYGIESWNSISNCSQTLSYDLTAVTLDLYHSNGYRARVRAVDGSRHSNWTVTNTRFSVDEVTLTVGSVNLEIHNGFILGKIQLPRPKMAPANDTYESIFSHFREYEIAIRKVPGNFTFTHKKVKHENFSLLTSGEVGEFCVQVKPSVASRSNKGMWSKEECISLTRQYFTVTNVIIFFAFVLLLSGALAYCLALQLYVRRRKKLPSVLLFKKPSPFIFISQRPSPETQDTIHPLDEEAFLKVSPELKNLDLHGSTDSGFGSTKPSLQTEEPQFLLPDPHPQADRTLGNREPPVLGDSCSSGSSNSTDSGICLQEPSLSPSTGPTWEQQVGSNSRGQDDSGIDLVQNSEGRAGDTQGGSALGHHSPPEPEVPGEEDPAAVAFQGYLRQTRCAEEKATKTGCLEEESPLTDGLGPKFGRCLVDEAGLHPPALAKGYLKQDPLEMTLASSGAPTGQWNQPTEEWSLLALSSCSDLGISDWSFAHDLAPLGCVAAPGGLLGSFNSDLVTLPLISSLQSSE

SEQ ID NO: 2 - protein, 235 aa, unidentified
MLPCLVVLLAALLSLRLGSDAHGTELPSPPSVWFEAEFFHHILHWTPIPNQSESTCYEVALLRYGIESWNSISNCSQTLSYDLTAVTLDLYHSNGYRARVRAVDGSRHSNWTVTNTRFSVDEVTLTVGSVNLEIHNGFILGKIQLPRPKMAPANDTYEGIFSHFREYEIAIRKVPGNFTFTHKKVKHENFSLLTSGEVGEFCVQVKPSVASRSNKGMWSKEECISLTRQYFTVTN

SEQ ID NO: 3 - protein, 214 aa, unidentified
HGTELPSPPSVWFEAEFFHHILHWTPIPNQSESTCYEVALLRYGIESWNSISNCSQTLSYDLTAVTLDLYHSNGYRARVRAVDGSRHSNWTVTNTRFSVDEVTLTVGSVNLEIHNGFILGKIQLPRPKMAPANDTYEGIFSHFREYEIAIRKVPGNFTFTHKKVKHENFSLLTSGEVGEFCVQVKPSVASRSNKGMWSKEECISLTRQYFTVTN

SEQ ID NO: 4 - protein, 209 aa, unidentified
HGTELPSPPSVWFEAEFFHHILHWTPIPNQSESTCYEVALLRYGIESWNSISNCSQTLSYDLTAVTLDLYHSNGYRARVRAVDGSRHSNWTVTNTRFSVDEVTLTVGSVNLEIHNGFILGKIQLPRPKMAPANDTYEGIFSHFREYEIAIRKVPGNFTFTHKKVKHENFSLLTSGEVGEFCVQVKPSVASRSNKGMWSKEECISLTRQY